European Patent Application EP 4 134 097 A1, published February 15, 2023. Title: Agent for inhibiting secretion of extracellular vesicle from cancer cells, therapeutic agent for cancer, and use thereof. Applicant: Theoria Science, Inc. The sequence listing filed with the application follows.

SEQUENCE LISTING (2 sequences)

SEQ ID NO: 1 - RNA, 21 nt, Artificial Sequence
  miRNA for PSAT1
  miR-891b (1)..(21)
gcaacuuaccugagucauuga

SEQ ID NO: 2 - RNA, 22 nt, Homo sapiens
  3'UTR (1)..(22)
uggacuuaauaaugcaaguugc